European Patent Specification EP 3 818 179 B1, published July 19, 2023. Title: Epigenetic method to detect and distinguish IPEX and IPEX-like syndromes, in particular in newborns. Applicant: Epiontis GmbH. The sequence listing filed with the application follows.

SEQUENCE LISTING (13 sequences)

SEQ ID NO: 1 - DNA, 20 bp, Homo sapiens
tgtttgggggtagaggattt

SEQ ID NO: 2 - DNA, 20 bp, Homo sapiens
tatcaccccacctaaaccaa

SEQ ID NO: 3 - DNA, 22 bp, Homo sapiens
aaatcctaaaatctcaaaacca

SEQ ID NO: 4 - DNA, 21 bp, Homo sapiens
ggtgatgatggaggtatgtta

SEQ ID NO: 5 - DNA, 23 bp, Homo sapiens
atggtggttggatgtgttgggtt

SEQ ID NO: 6 - DNA, 18 bp, Homo sapiens
atggcggtcggatgcgtc

SEQ ID NO: 7 - DNA, 336 bp, Homo sapiens
tgtctgggggtagaggacctagagggccgggctgggcagccggcttcctgcactgtctgttgggacgtccctttctgactgggtttctcagaagctgaatgggggatgtttctgggacacagattatgttttcatatcggggtctgcatctgggccctgttgtcacagcccccgacttgcccagatttttccgccattgacgtcatggcggccggatgcgccgggcttcatcgacaccacggaggaagagaagagggcagataccccaccccacaggtttcgttccgagaactggctgccctgtcctgcagcaggcttggcccaggtggggtgaca

SEQ ID NO: 8 - DNA, 22 bp, Homo sapiens
ggtttttggtattgtaggtttt

SEQ ID NO: 9 - DNA, 21 bp, Homo sapiens
ccaattacaacataacaacca

SEQ ID NO: 10 - DNA, 29 bp, Homo sapiens
tgtttggatgttgtgtttgtggtagagtg

SEQ ID NO: 11 - DNA, 22 bp, Homo sapiens
ggttttgtgtatgttaggtttg

SEQ ID NO: 12 - DNA, 22 bp, Homo sapiens
ccacattacaacataaacacac

SEQ ID NO: 13 - DNA, 29 bp, Homo sapiens
tgttgtgatgttggttttggtgtagaggt